European Patent Application EP 4 624 578 A1, published October 1, 2025. Title: Fusion gene containing encoding gene of chimeric antigen receptor and encoding gene of chimeric switch receptor and use thereof. Applicant: Carbiogene therapeutics Co, Ltd. Application CN WO2024/108614A1, filed November 28, 2022. The sequence listing filed with the application follows.

SEQUENCE LISTING (8 sequences)

SEQ ID NO: 1 - protein, 406 aa, synthetic construct
MGRGLLRGLWPLHIVLWTRIASTIPPHVQKSVNNDMIVTDNNGAVKFPQLCKFCDVRFSTCDNQKSCMSNCSITSICEKPQEVCVAVWRKNDENITLETVCHDPKLPYHDFILEDAASPKCIMKEKKKPGETFFMCSCSSDECNDNIIFSEEYNTSNPDLLLVIFQGIQAEAAAKEAAAKEAAAKALDSPDRPWNPPTFSPALLVVTEGDNATFTCSFSNTSESFHVVWHRESPSGQTDTLAAFPEDRSQPGQDCRFRVTQLPNGRDFHMSVVRARRNDSGTYVCGVISLAPKIQIKESLRAELRVTERRAEVPTAHPSPSPRPAGQFQTLVSDFIRILVIFSGMFLVFTLAGALFLHQRRKYRSNKGESPVEPAEPCRYSCPREEEGSTIPIQEDYRKPEPACSP

SEQ ID NO: 2 - DNA, 1221 bp, synthetic construct
  source 1..1221: mol_type = other DNA
atgggtcgggggctgctcaggggcctgtggccgctgcacatcgtcctgtggacgcgtatcgccagcacgatcccaccgcacgttcagaagtcggttaataacgacatgatagtcactgacaacaacggtgcagtcaagtttccacaactgtgtaaattttgtgatgtgagattttccacctgtgacaaccagaaatcctgcatgagcaactgcagcatcacctccatctgtgagaagccacaggaagtctgtgtggctgtatggagaaagaatgacgagaacataacactagagacagtttgccatgaccccaagctcccctaccatgactttattctggaagatgctgcttctccaaagtgcattatgaaggaaaaaaaaaagcctggtgagactttcttcatgtgttcctgtagctctgatgagtgcaatgacaacatcatcttctcagaagaatataacaccagcaatcctgacttgttgctagtcatatttcaagggattcaagccgaagcagcagcaaaggaggccgcagcgaaggaagcagctgcgaaggccctagactccccagacaggccctggaacccccccaccttctccccagccctgctcgtggtgaccgaaggggacaacgccaccttcacctgcagcttctccaacacatcggagagcttccacgtcgtgtggcaccgcgagagccccagcggacagacggacacactggccgccttccccgaggaccgcagccagcccggccaggactgccgcttccgtgtcacacaactgcccaacgggcgtgacttccacatgagcgtggtcagggcccggcgcaatgacagcggcacctacgtgtgtggggtcatctccctggcccccaagatccagatcaaagagagcctgcgggcagagctcagggtgacagagagaagggcagaagtgcccacagcccaccccagcccctcacccaggccagccggccagttccaaaccctggtgagcgactttatcagaatcctggtgatcttctctggcatgttcctggtgtttacactggccggcgccctgtttctgcaccagagacgcaagtaccgcagcaacaagggagaaagccccgtggagcccgctgagccctgcagatactcctgccccagagaggaggagggcagcaccattcccatccaggaggactacagaaaacccgagcccgcctgcagcccatga

SEQ ID NO: 3 - DNA, 3882 bp, synthetic construct
  source 1..3882: mol_type = other DNA
atggctctgcctgtgaccgccctgctgctgcctctggctctgctgctgcacgccgctcggcctgacgtggtgatgacccagagccccctgagcctgcccgtgaccccaggagaacccgccagcattagctgcagaagcagccagagcctggtgcacagcaacagaaacacctatctgcactggtatctgcagaaaccaggacagagcccccagctgctgatctacaaagtgagcaatagattcagcggggtgcccgacagattcagcggctcaggaagcggaaccgactttaccctgaagattagcagagtggaggctgaggacgtgggcgtgtactactgcagccagaacacccacgtgccacctacctttggacagggcaccaaactggagatcaagggcggcgggggaagcggcggaggaggaagcggaggaggaggaagtcaggtgcagctggtgcagagcggcgccgaggtgaaaaagccaggcgcaagcgtgaaggtgagctgcaaggcaagcggatacacattcacagactacgagatgcattgggtgaggcaggcacccggccaggggctggaatggatgggagcactggaccccaagacaggcgacacagcctacagccagaagttcaagggcagagtgaccctgaccgccgacaaaagcaccagcacagcctatatggaactgagcagcctgaccagcgaggacaccgccgtgtactactgtacccggttttacagctacacctactggggacagggcacactggtgaccgtgagcagcactacaactccagcacccagaccccctacacctgctccaactatcgcaagtcagcccctgtcactgcgccctgaagcctgtcgccctgctgccgggggagctgtgcatactcggggactggactttgcctgtgatatctacatctgggcgcccttggccgggacttgtggggtccttctcctgtcactggttatcaccctttactgcaggttcagtgtcgtgaagagaggccggaagaagctgctgtacatcttcaagcagcctttcatgaggcccgtgcagactacccaggaggaagatggatgcagctgtagattccctgaagaggaggaaggaggctgtgagctgagagtgaagttctcccgaagcgcagatgccccagcctatcagcagggacagaatcagctgtacaacgagctgaacctgggaagacgggaggaatacgatgtgctggacaaaaggcggggcagagatcctgagatgggcggcaaaccaagacggaagaacccccaggaaggtctgtataatgagctgcagaaagacaagatggctgaggcctactcagaaatcgggatgaagggcgaaagaaggagaggaaaaggccacgacggactgtaccaggggctgagtacagcaacaaaagacacctatgacgctctgcacatgcaggctctgccaccaagacgagctaaacgaggctcaggcgcgacgaactttagtttgctgaagcaagctggggatgtagaggaaaatccgggtcccatggccctgaccttcgccctgctggtggccctgctggtcctgagctgcaagagctcctgcagcgtggggtgcgacctgccccagacccacagcctgggctccagaagaaccctgatgctgctggcccagatgagaagaatcagtctgttcagctgcctgaaagacagacacgactttggcttccctcaggaggaatttggaaaccagttccagaaggccgaaaccatccccgtgctgcacgagatgatccagcagatcttcaacctgttctccaccaaagatagcagcgcagcctgggacgaaaccctgctggacaagttctacaccgagctgtaccagcagctgaacgacctggaggcctgcgtgatccagggcgtgggagtgaccgagacaccactgatgaaagaggatagcattctggccgtgaggaaatacttccagagaatcaccctgtacctgaaagagaaaaagtacagtccctgcgcctgggaggtggtgagagccgagatcatgagaagcttcagcctgagcaccaatctgcaggaaagcctgagaagcaaggagtgagaattcttgtagataccgggtaggggaggcgcttttcccaaggcagtctggagcatgcgctttagcagccccgctgggcacttggcgctacacaagtggcctctggcctcgcacacattccacatccaccggtaggcgccaaccggctccgttctttggtggccccttcgcgccaccttctactcctcccctagtcaggaagttcccccccgccccgcagctcgcgtcgtgcaggacgtgacaaatggaagtagcacgtctcactagtctcgtgcagatggacagcaccgctgagcaatggaagcgggtaggcctttggggcagcggccaatagcagctttgctccttcgctttctgggctcagaggctgggaaggggtgggtccgggggcgggctcaggggcgggctcaggggcggggcgggcgcccgaaggtcctccggaggcccggcattctgcacgcttcaaaagcgcacgtctgccgcgctgttctcctcttcctcatctccgggcctttcgaccagttaactccaccggtcgccaccatgggtcgggggctgctcaggggcctgtggccgctgcacatcgtcctgtggacgcgtatcgccagcacgatcccaccgcacgttcagaagtcggttaataacgacatgatagtcactgacaacaacggtgcagtcaagtttccacaactgtgtaaattttgtgatgtgagattttccacctgtgacaaccagaaatcctgcatgagcaactgcagcatcacctccatctgtgagaagccacaggaagtctgtgtggctgtatggagaaagaatgacgagaacataacactagagacagtttgccatgaccccaagctcccctaccatgactttattctggaagatgctgcttctccaaagtgcattatgaaggaaaaaaaaaagcctggtgagactttcttcatgtgttcctgtagctctgatgagtgcaatgacaacatcatcttctcagaagaatataacaccagcaatcctgacttgttgctagtcatatttcaagggattcaagccgaagcagcagcaaaggaggccgcagcgaaggaagcagctgcgaaggccctagactccccagacaggccctggaacccccccaccttctccccagccctgctcgtggtgaccgaaggggacaacgccaccttcacctgcagcttctccaacacatcggagagcttccacgtcgtgtggcaccgcgagagccccagcggacagacggacacactggccgccttccccgaggaccgcagccagcccggccaggactgccgcttccgtgtcacacaactgcccaacgggcgtgacttccacatgagcgtggtcagggcccggcgcaatgacagcggcacctacgtgtgtggggtcatctccctggcccccaagatccagatcaaagagagcctgcgggcagagctcagggtgacagagagaagggcagaagtgcccacagcccaccccagcccctcacccaggccagccggccagttccaaaccctggtgagcgactttatcagaatcctggtgatcttctctggcatgttcctggtgtttacactggccggcgccctgtttctgcaccagagacgcaagtaccgcagcaacaagggagaaagccccgtggagcccgctgagccctgcagatactcctgccccagagaggaggagggcagcaccattcccatccaggaggactacagaaaacccgagcccgcctgcagcccatga

SEQ ID NO: 4 - protein, 491 aa, synthetic construct
MALPVTALLLPLALLLHAARPDVVMTQSPLSLPVTPGEPASISCRSSQSLVHSNRNTYLHWYLQKPGQSPQLLIYKVSNRFSGVPDRFSGSGSGTDFTLKISRVEAEDVGVYYCSQNTHVPPTFGQGTKLEIKGGGGSGGGGSGGGGSQVQLVQSGAEVKKPGASVKVSCKASGYTFTDYEMHWVRQAPGQGLEWMGALDPKTGDTAYSQKFKGRVTLTADKSTSTAYMELSSLTSEDTAVYYCTRFYSYTYWGQGTLVTVSSTTTPAPRPPTPAPTIASQPLSLRPEACRPAAGGAVHTRGLDFACDIYIWAPLAGTCGVLLLSLVITLYCRFSVVKRGRKKLLYIFKQPFMRPVQTTQEEDGCSCRFPEEEEGGCELRVKFSRSADAPAYQQGQNQLYNELNLGRREEYDVLDKRRGRDPEMGGKPRRKNPQEGLYNELQKDKMAEAYSEIGMKGERRRGKGHDGLYQGLSTATKDTYDALHMQALPPR

SEQ ID NO: 5 - protein, 188 aa, synthetic construct
MALTFALLVALLVLSCKSSCSVGCDLPQTHSLGSRRTLMLLAQMRRISLFSCLKDRHDFGFPQEEFGNQFQKAETIPVLHEMIQQIFNLFSTKDSSAAWDETLLDKFYTELYQQLNDLEACVIQGVGVTETPLMKEDSILAVRKYFQRITLYLKEKKYSPCAWEVVRAEIMRSFSLSTNLQESLRSKE

SEQ ID NO: 6 - protein, 21 aa, synthetic construct
VKQTLNFDLLKLAGCVESNPG

SEQ ID NO: 7 - protein, 17 aa, synthetic construct
EGRGSLLTCGDVEENPG

SEQ ID NO: 8 - protein, 19 aa, synthetic construct
QCTNYALLKLAGDVESNPG